European Patent Application EP 4 209 211 A1, published July 12, 2023. Title: Surtuin activating agent and method for activating surtuin. Applicant: YUKI GOSEI KOGYO CO., LTD. KYUSYU UNIVERSITY, NATIONAL UNIVERSITY CORPORATION. The sequence listing filed with the application follows.

SEQUENCE LISTING (12 sequences)

SEQ ID NO: 1 - DNA, 19 bp, Artificial Sequence
  beta-actin  forward primer
ggccaggtcatcactattg

SEQ ID NO: 2 - DNA, 21 bp, Artificial Sequence
  beta-actin  reverse primer
gaggtctttacggatgtcaac

SEQ ID NO: 3 - DNA, 24 bp, Artificial Sequence
  Sirt1 forward primer
gcagacgtggtaatgtccaaacag

SEQ ID NO: 4 - DNA, 25 bp, Artificial Sequence
  Sirt1 reverse primer
acatcttggcagtatttgtggtgaa

SEQ ID NO: 5 - DNA, 21 bp, Artificial Sequence
  Sirt3 forward primer
atgcacggtctgtcgaaggtc

SEQ ID NO: 6 - DNA, 24 bp, Artificial Sequence
  Sirt3 reverse primer
agaacacaatgtcgggtttcacaa

SEQ ID NO: 7 - DNA, 24 bp, Artificial Sequence
  Human Sirt1 forward
gcctcacatgcaagctctagtgac

SEQ ID NO: 8 - DNA, 24 bp, Artificial Sequence
  Human Sirt1 reverse
ttcgaggatctgtgccaatcataa

SEQ ID NO: 9 - DNA, 24 bp, Artificial Sequence
  Human Sirt3 forward
agccctcttcatgttccgaagtgt

SEQ ID NO: 10 - DNA, 24 bp, Artificial Sequence
  Human Sirt3 reverse
tcatgtcaacacctgcagtccctt

SEQ ID NO: 11 - DNA, 17 bp, Artificial Sequence
  Sirt6 forward
aattacgcggcggggct

SEQ ID NO: 12 - DNA, 17 bp, Artificial Sequence
  Sirt6 reverse
cgcgcgctctcaaaggt